European Patent Application EP 4 702 992 A1, published March 4, 2026. Title: ANTIBODY-DRUG CONJUGATE. Applicant: CSPC MEGALITH BIOPHARMACEUTICAL CO., LTD. Application CN. The sequence listing filed with the application follows.

SEQUENCE LISTING (44 sequences)

SEQ ID NO: 1 - protein, 5 aa, synthetic construct
DYFMN

SEQ ID NO: 2 - protein, 17 aa, synthetic construct
DVNPKTGSPSYNQKFKG

SEQ ID NO: 3 - protein, 10 aa, synthetic construct
RYGFLYSMDY

SEQ ID NO: 4 - protein, 11 aa, synthetic construct
RASQDISNYLN

SEQ ID NO: 5 - protein, 7 aa, synthetic construct
YTSRLHS

SEQ ID NO: 6 - protein, 9 aa, synthetic construct
QQGNTHPFT

SEQ ID NO: 7 - protein, 119 aa, synthetic construct
QVQLVQSGAEVKKPGASVKVSCKASGYTFTDYFMNWVRQAPGQGLEWMGDVNPKTGSPSYNQKFKGRVTMTRDTSTSTVYMELSSLRSEDTAVYYCARRYGFLYSMDYWGQGTSVTVSS

SEQ ID NO: 8 - protein, 107 aa, synthetic construct
DIQMTQSPSSLSASVGDRVTITCRASQDISNYLNWYQQKPGKAVKVLIYYTSRLHSGVPSRFSGSGSGTDFTFTISSLQPEDIATYYCQQGNTHPFTFGGGTKVEIK

SEQ ID NO: 9 - protein, 449 aa, synthetic construct
QVQLVQSGAEVKKPGASVKVSCKASGYTFTDYFMNWVRQAPGQGLEWMGDVNPKTGSPSYNQKFKGRVTMTRDTSTSTVYMELSSLRSEDTAVYYCARRYGFLYSMDYWGQGTSVTVSSASTKGPSVFPLAPSSKSTSGGTAALGCLVKDYFPEPVTVSWNSGALTSGVHTFPAVLQSSGLYSLSSVVTVPSSSLGTQTYICNVNHKPSNTKVDKRVEPKSCDKTHTCPPCPAPEAAGGPSVFLFPPKPKDTLMISRTPEVTCVVVDVSHEDPEVKFNWYVDGVEVHNAKTKPREEQYNSTYRVVSVLTVLHQDWLNGKEYKCKVSNKALAASIEKTISKAKGQPREPQVYTLPPSREEMTKNQVSLTCLVKGFYPSDIAVEWESNGQPENNYKTTPPVLDSDGSFFLYSKLTVDKSRWQQGNVFSCSVMHEALHNHYTQKSLSLSPGK

SEQ ID NO: 10 - protein, 449 aa, synthetic construct
QVQLVQSGAEVKKPGASVKVSCKASGYTFTDYFMNWVRQAPGQGLEWMGDVNPKTGSPSYNQKFKGRVTMTRDTSTSTVYMELSSLRSEDTAVYYCARRYGFLYSMDYWGQGTSVTVSSASTKGPSVFPLAPSSKSTSGGTAALGCLVKDYFPEPVTVSWNSGALTSGVHTFPAVLQSSGLYSLSSVVTVPSSSLGTQTYICNVNHKPSNTKVDKRVEPKSCDKTHTSPPCPAPEAAGGPSVFLFPPKPKDTLMISRTPEVTCVVVDVSHEDPEVKFNWYVDGVEVHNAKTKPREEQYNSTYRVVSVLTVLHQDWLNGKEYKCKVSNKALAASIEKTISKAKGQPREPQVYTLPPSREEMTKNQVSLTCLVKGFYPSDIAVEWESNGQPENNYKTTPPVLDSDGSFFLYSKLTVDKSRWQQGNVFSCSVMHEALHNHYTQKSLSLSPGK

SEQ ID NO: 11 - protein, 214 aa, synthetic construct
DIQMTQSPSSLSASVGDRVTITCRASQDISNYLNWYQQKPGKAVKVLIYYTSRLHSGVPSRFSGSGSGTDFTFTISSLQPEDIATYYCQQGNTHPFTFGGGTKVEIKRTVAAPSVFIFPPSDEQLKSGTASVVCLLNNFYPREAKVQWKVDNALQSGNSQESVTEQDSKDSTYSLSSTLTLSKADYEKHKVYACEVTHQGLSSPVTKSFNRGEC

SEQ ID NO: 12 - protein, 5 aa, synthetic construct
DYYMK

SEQ ID NO: 13 - protein, 17 aa, synthetic construct
AFNLNNGDTFYNQKFKG

SEQ ID NO: 14 - protein, 8 aa, synthetic construct
DVYGYGDY

SEQ ID NO: 15 - protein, 15 aa, synthetic construct
RASKSVSTSGYSYMH

SEQ ID NO: 16 - protein, 7 aa, synthetic construct
LASNLDS

SEQ ID NO: 17 - protein, 9 aa, synthetic construct
QHSRELPYT

SEQ ID NO: 18 - protein, 117 aa, synthetic construct
QVQLVQSGAEVKKPGASVKVSCKASGYTFTDYYMKWVRQAPGQRLEWMGAFNLNNGDTFYNQKFKGRVTITRDTSASTAYMELSSLRSEDTAVYYCARDVYGYGDYWGQGTSVTVSS

SEQ ID NO: 19 - protein, 111 aa, synthetic construct
DIVMTQSPDSLAVSLGERATINCRASKSVSTSGYSYMHWYQQKPGQPPKLLIYLASNLDSGVPDRFSGSGSGTDFTLTISSLQAEDVAVYYCQHSRELPYTFGGGTKLEIK

SEQ ID NO: 20 - protein, 447 aa, synthetic construct
QVQLVQSGAEVKKPGASVKVSCKASGYTFTDYYMKWVRQAPGQRLEWMGAFNLNNGDTFYNQKFKGRVTITRDTSASTAYMELSSLRSEDTAVYYCARDVYGYGDYWGQGTSVTVSSASTKGPSVFPLAPSSKSTSGGTAALGCLVKDYFPEPVTVSWNSGALTSGVHTFPAVLQSSGLYSLSSVVTVPSSSLGTQTYICNVNHKPSNTKVDKKVEPKSCDKTHTCPPCPAPEAAGGPSVFLFPPKPKDTLMISRTPEVTCVVVDVSHEDPEVKFNWYVDGVEVHNAKTKPREEQYNSTYRVVSVLTVLHQDWLNGKEYKCKVSNKALAASIEKTISKAKGQPREPQVYTLPPSRDELTKNQVSLTCLVKGFYPSDIAVEWESNGQPENNYKTTPPVLDSDGSFFLYSKLTVDKSRWQQGNVFSCSVMHEALHNHYTQKSLSLSPGK

SEQ ID NO: 21 - protein, 218 aa, synthetic construct
DIVMTQSPDSLAVSLGERATINCRASKSVSTSGYSYMHWYQQKPGQPPKLLIYLASNLDSGVPDRFSGSGSGTDFTLTISSLQAEDVAVYYCQHSRELPYTFGGGTKLEIKRTVAAPSVFIFPPSDEQLKSGTASVVCLLNNFYPREAKVQWKVDNALQSGNSQESVTEQDSKDSTYSLSSTLTLSKADYEKHKVYACEVTHQGLSSPVTKSFNRGEC

SEQ ID NO: 22 - protein, 5 aa, synthetic construct
GYGLS

SEQ ID NO: 23 - protein, 17 aa, synthetic construct
MISSGGSYTYYADSVKG

SEQ ID NO: 24 - protein, 10 aa, synthetic construct
HGDDPAWFAY

SEQ ID NO: 25 - protein, 12 aa, synthetic construct
SVSSSISSNNLH

SEQ ID NO: 26 - protein, 7 aa, synthetic construct
GTSNLAS

SEQ ID NO: 27 - protein, 11 aa, synthetic construct
QQWSSYPYMYT

SEQ ID NO: 28 - protein, 119 aa, synthetic construct
EVQLVESGGGVVQPGRSLRLSCSASGFTFSGYGLSWVRQAPGKGLEWVAMISSGGSYTYYADSVKGRFAISRDNAKNTLFLQMDSLRPEDTGVYFCARHGDDPAWFAYWGQGTPVTVSS

SEQ ID NO: 29 - protein, 110 aa, synthetic construct
DIQLTQSPSSLSASVGDRVTITCSVSSSISSNNLHWYQQKPGKAPKPWIYGTSNLASGVPSRFSGSGSGTDYTFTISSLQPEDIATYYCQQWSSYPYMYTFGQGTKVEIK

SEQ ID NO: 30 - protein, 449 aa, synthetic construct
EVQLVESGGGVVQPGRSLRLSCSASGFTFSGYGLSWVRQAPGKGLEWVAMISSGGSYTYYADSVKGRFAISRDNAKNTLFLQMDSLRPEDTGVYFCARHGDDPAWFAYWGQGTPVTVSSASTKGPSVFPLAPSSKSTSGGTAALGCLVKDYFPEPVTVSWNSGALTSGVHTFPAVLQSSGLYSLSSVVTVPSSSLGTQTYICNVNHKPSNTKVDKKVEPKSCDKTHTCPPCPAPELLGGPSVFLFPPKPKDTLMISRTPEVTCVVVDVSHEDPEVKFNWYVDGVEVHNAKTKPREEQYNSTYRVVSVLTVLHQDWLNGKEYKCKVSNKALPAPIEKTISKAKGQPREPQVYTLPPSRDELTKNQVSLTCLVKGFYPSDIAVEWESNGQPENNYKTTPPVLDSDGSFFLYSKLTVDKSRWQQGNVFSCSVMHEALHNHYTQKSLSLSPGK

SEQ ID NO: 31 - protein, 217 aa, synthetic construct
DIQLTQSPSSLSASVGDRVTITCSVSSSISSNNLHWYQQKPGKAPKPWIYGTSNLASGVPSRFSGSGSGTDYTFTISSLQPEDIATYYCQQWSSYPYMYTFGQGTKVEIKRTVAAPSVFIFPPSDEQLKSGTASVVCLLNNFYPREAKVQWKVDNALQSGNSQESVTEQDSKDSTYSLSSTLTLSKADYEKHKVYACEVTHQGLSSPVTKSFNRGEC

SEQ ID NO: 32 - protein, 449 aa, synthetic construct
EVQLVESGGGVVQPGRSLRLSCSASGFTFSGYGLSWVRQAPGKGLEWVAMISSGGSYTYYADSVKGRFAISRDNAKNTLFLQMDSLRPEDTGVYFCARHGDDPAWFAYWGQGTPVTVSSASTKGPSVFPLAPSSKSTSGGTAALGCLVKDYFPEPVTVSWNSGALTSGVHTFPAVLQSSGLYSLSSVVTVPSSSLGTQTYICNVNHKPSNTKVDKKVEPKSCDKTHTCPPCPAPEAAGGPSVFLFPPKPKDTLMISRTPEVTCVVVDVSHEDPEVKFNWYVDGVEVHNAKTKPREEQYNSTYRVVSVLTVLHQDWLNGKEYKCKVSNKALAASIEKTISKAKGQPREPQVYTLPPSRDELTKNQVSLTCLVKGFYPSDIAVEWESNGQPENNYKTTPPVLDSDGSFFLYSKLTVDKSRWQQGNVFSCSVMHEALHNHYTQKSLSLSPGK

SEQ ID NO: 33 - protein, 450 aa, synthetic construct
EVQLVESGGGLVQPGGSLRLSCAASGFNIKDTYIHWVRQAPGKGLEWVARIYPTNGYTRYADSVKGRFTISADTSKNTAYLQMNSLRAEDTAVYYCSRWGGDGFYAMDYWGQGTLVTVSSASTKGPSVFPLAPSSKSTSGGTAALGCLVKDYFPEPVTVSWNSGALTSGVHTFPAVLQSSGLYSLSSVVTVPSSSLGTQTYICNVNHKPSNTKVDKKVEPKSCDKTHTCPPCPAPELLGGPSVFLFPPKPKDTLMISRTPEVTCVVVDVSHEDPEVKFNWYVDGVEVHNAKTKPREEQYNSTYRVVSVLTVLHQDWLNGKEYKCKVSNKALPAPIEKTISKAKGQPREPQVYTLPPSREEMTKNQVSLTCLVKGFYPSDIAVEWESNGQPENNYKTTPPVLDSDGSFFLYSKLTVDKSRWQQGNVFSCSVMHEALHNHYTQKSLSLSPGK

SEQ ID NO: 34 - protein, 214 aa, synthetic construct
DIQMTQSPSSLSASVGDRVTITCRASQDVNTAVAWYQQKPGKAPKLLIYSASFLYSGVPSRFSGSRSGTDFTLTISSLQPEDFATYYCQQHYTTPPTFGQGTKVEIKRTVAAPSVFIFPPSDEQLKSGTASVVCLLNNFYPREAKVQWKVDNALQSGNSQESVTEQDSKDSTYSLSSTLTLSKADYEKHKVYACEVTHQGLSSPVTKSFNRGEC

SEQ ID NO: 35 - protein, 120 aa, synthetic construct [sequence omitted]

SEQ ID NO: 36 - protein, 107 aa, synthetic construct [sequence omitted]

SEQ ID NO: 37 - protein, 5 aa, synthetic construct
DTYIH

SEQ ID NO: 38 - protein, 17 aa, synthetic construct
RIYPTNGYTRYADSVKG

SEQ ID NO: 39 - protein, 11 aa, synthetic construct
WGGDGFYAMDY

SEQ ID NO: 40 - protein, 11 aa, synthetic construct
RASQDVNTAVA

SEQ ID NO: 41 - protein, 7 aa, synthetic construct
SASFLYS

SEQ ID NO: 42 - protein, 9 aa, synthetic construct
QQHYTTPPT

SEQ ID NO: 43 - protein, 452 aa, synthetic construct
QVQLVQSGAEVKKPGSSVKVSCKASGYTFTNYVMHWVRQAPGQGLEWMGYINPYNDDVKYNEKFKGRVTITADESTSTAYMELSSLRSEDTAVYYCARWGYYGSPLYYFDYWGQGTLVTVSSASTKGPSVFPLAPSSKSTSGGTAALGCLVKDYFPEPVTVSWNSGALTSGVHTFPAVLQSSGLYSLSSVVTVPSSSLGTQTYICNVNHKPSNTKVDKRVEPKSCDKTHTCPPCPAPELLGGPSVFLFPPKPKDTLMISRTPEVTCVVVDVSHEDPEVKFNWYVDGVEVHNAKTKPREEQYNSTYRVVSVLTVLHQDWLNGKEYKCKVSNKALPAPIEKTISKAKGQPREPQVYTLPPSREEMTKNQVSLTCLVKGFYPSDIAVEWESNGQPENNYKTTPPVLDSDGSFFLYSKLTVDKSRWQQGNVFSCSVMHEALHNHYTQKSLSLSPGK

SEQ ID NO: 44 - protein, 213 aa, synthetic construct
EIVLTQSPATLSLSPGERATLSCRASSRLIYMHWYQQKPGQAPRPLIYATSNLASGIPARFSGSGSGTDFTLTISSLEPEDFAVYYCQQWNSNPPTFGQGTKVEIKRTVAAPSVFIFPPSDEQLKSGTASVVCLLNNFYPREAKVQWKVDNALQSGNSQESVTEQDSKDSTYSLSSTLTLSKADYEKHKVYACEVTHQGLSSPVTKSFNRGEC